European Patent Application EP 4 474 383 A2, published December 11, 2024. Title: APOPTOSIS-INDUCING AGENTS FOR THE TREATMENT OF CANCER AND IMMUNE AND AUTOIMMUNE DISEASES. Applicant: AbbVie Ireland Unlimited Company. Application EP 24195253.0, filed May 26, 2010. The sequence listing filed with the application follows.

SEQUENCE LISTING (1 sequence)

SEQ ID NO: 1 - protein, 16 aa, synthetic construct
  REGION 1..16: note = Probe Peptide
  MOD_RES 1: note = Gly is modified with acetyl
  MOD_RES 13: note = Lys is modified with 6-FAM
  MOD_RES 16: note = Arg is modified with NH2
GQVGRQLAIIGDKINR